European Patent Application EP 4 410 308 A1, published August 7, 2024. Title: CYTOTOXICITY-INDUCING THERAPEUTIC AGENT FOR TREATING CANCER. Applicant: CHUGAI SEIYAKU KABUSHIKI KAISHA. The sequence listing filed with the application follows.

SEQUENCE LISTING (215 sequences)

SEQ ID NO: 1 - protein, 119 aa, synthetic construct
  REGION 1..119: note = an artificially synthesized sequence
QVQLVESGGGVVQPGGSLRLSCAASGFTFSSYTMSWVRQAPGQGLEWMGTISSGGGRTYYPDSVKGRFTISRDNSKNTLYLQMNSLRDEDTAVYYCARGDYRYDGFAYWGEGTLVTVSS

SEQ ID NO: 2 - protein, 119 aa, synthetic construct
  REGION 1..119: note = an artificially synthesized sequence
QVQLVESGGGVVQPGGSLRLSCAASGFTFSSYTMSWVREAPGQGLEWMGTISSGGGRTYYPDSVKGRFTISRDNSKNTLYLQMNSLRDEDTAVYYCARGDYRYDGFAYWGEGTLVTVSS

SEQ ID NO: 3 - protein, 128 aa, synthetic construct
  REGION 1..128: note = an artificially synthesized sequence
QVQLVESGGGLVQPGRSLRLSCAASGFKFSNVWFHWVRKAPGKGLEWVAQIKDYYNAYAAYYAPSVKGRFTISRDDSKNSIYLQMNSLKTEDTAVYYCHYVHYASASTLLPAEGVDAWGQGTTVTVSS

SEQ ID NO: 4 - protein, 128 aa, synthetic construct
  REGION 1..128: note = an artificially synthesized sequence
QVQLVESGGGLVQPGRSLRLSCAASGFKFSNVWFHWVRKAPGKGLEWVAQIKDYYNAYAGYYHPSVKGRFTISRDDSKNSIYLQMNSLKTEDTAVYYCHYVHYAAASQLLPAEGVDAWGQGTTVTVSS

SEQ ID NO: 5 - protein, 128 aa, synthetic construct
  REGION 1..128: note = an artificially synthesized sequence
QVQLVESGGGLVQPGRSLRLSCAASGFKFSNVWFHWVRQAPGKGLEWVAQIKDYYNAYAAYYAPSVKGRFTISRDDSKNSIYLQMNSLKTEDTAVYYCHYVHYASASTLLPAEGVDAWGQGTTVTVSS

SEQ ID NO: 6 - protein, 128 aa, synthetic construct
  REGION 1..128: note = an artificially synthesized sequence
QVQLVESGGGLVQPGRSLRLSCAASGFKFSNVWFHWVRQAPGKGLEWVAQIKDYYNAYAGYYHPSVKGRFTISRDDSKNSIYLQMNSLKTEDTAVYYCHYVHYAAASQLLPAEGVDAWGQGTTVTVSS

SEQ ID NO: 7 - protein, 5 aa, synthetic construct
  REGION 1..5: note = an artificially synthesized sequence
SYTMS

SEQ ID NO: 8 - protein, 5 aa, synthetic construct
  REGION 1..5: note = an artificially synthesized sequence
SYTMS

SEQ ID NO: 9 - protein, 5 aa, synthetic construct
  REGION 1..5: note = an artificially synthesized sequence
NVWFH

SEQ ID NO: 10 - protein, 5 aa, synthetic construct
  REGION 1..5: note = an artificially synthesized sequence
NVWFH

SEQ ID NO: 11 - protein, 5 aa, synthetic construct
  REGION 1..5: note = an artificially synthesized sequence
NVWFH

SEQ ID NO: 12 - protein, 5 aa, synthetic construct
  REGION 1..5: note = an artificially synthesized sequence
NVWFH

SEQ ID NO: 13 - protein, 17 aa, synthetic construct
  REGION 1..17: note = an artificially synthesized sequence
TISSGGGRTYYPDSVKG

SEQ ID NO: 14 - protein, 17 aa, synthetic construct
  REGION 1..17: note = an artificially synthesized sequence
TISSGGGRTYYPDSVKG

SEQ ID NO: 15 - protein, 19 aa, synthetic construct
  REGION 1..19: note = an artificially synthesized sequence
QIKDYYNAYAAYYAPSVKG

SEQ ID NO: 16 - protein, 19 aa, synthetic construct
  REGION 1..19: note = an artificially synthesized sequence
QIKDYYNAYAGYYHPSVKG

SEQ ID NO: 17 - protein, 19 aa, synthetic construct
  REGION 1..19: note = an artificially synthesized sequence
QIKDYYNAYAAYYAPSVKG

SEQ ID NO: 18 - protein, 19 aa, synthetic construct
  REGION 1..19: note = an artificially synthesized sequence
QIKDYYNAYAGYYHPSVKG

SEQ ID NO: 19 - protein, 10 aa, synthetic construct
  REGION 1..10: note = an artificially synthesized sequence
GDYRYDGFAY

SEQ ID NO: 20 - protein, 10 aa, synthetic construct
  REGION 1..10: note = an artificially synthesized sequence
GDYRYDGFAY

SEQ ID NO: 21 - protein, 17 aa, synthetic construct
  REGION 1..17: note = an artificially synthesized sequence
VHYASASTLLPAEGVDA

SEQ ID NO: 22 - protein, 17 aa, synthetic construct
  REGION 1..17: note = an artificially synthesized sequence
VHYAAASQLLPAEGVDA

SEQ ID NO: 23 - protein, 17 aa, synthetic construct
  REGION 1..17: note = an artificially synthesized sequence
VHYASASTLLPAEGVDA

SEQ ID NO: 24 - protein, 17 aa, synthetic construct
  REGION 1..17: note = an artificially synthesized sequence
VHYAAASQLLPAEGVDA

SEQ ID NO: 25 - protein, 107 aa, synthetic construct
  REGION 1..107: note = an artificially synthesized sequence
DIQMTQSPSSLSASVGDRVTITCRASYNIDSYLAWYQQKPGKAPELLIYYSTLLVDGVPDRFSGSRSGTDFTLTISSLQPEDFATYYCQHYYSIPYTFGQGTKVEIE

SEQ ID NO: 26 - protein, 107 aa, synthetic construct
  REGION 1..107: note = an artificially synthesized sequence
DIQMTQSPSSLSASVGDRVTITCRASYNIDSYLAWYQKKPGKAPELLIYYSTLLVDGVPDRFSGSRSGTDFTLTISSLQPEDFATYYCQHYYSIPYTFGQGTKVEIE

SEQ ID NO: 27 - protein, 112 aa, synthetic construct
  REGION 1..112: note = an artificially synthesized sequence
DIVMTQSPLSLPVTPGEPASISCQPSQEVVHMNRNTYLHWYQEKPGQAPRLLIYKVSNRFPGVPDRFSGSGSGTDFTLKISRVEAEDVGVYYCAQGTSHPFTFGQGTKLEIK

SEQ ID NO: 28 - protein, 112 aa, synthetic construct
  REGION 1..112: note = an artificially synthesized sequence
DIVMTQSPLSLPVTPGEPASISCQPSQEVVHMNRNTYLHWYQQKPGQAPRLLIYKVSNRFPGVPDRFSGSGSGTDFTLKISRVEAEDVGVYYCAQGTSHPFTFGQGTKLEIK

SEQ ID NO: 29 - protein, 11 aa, synthetic construct
  REGION 1..11: note = an artificially synthesized sequence
RASYNIDSYLA

SEQ ID NO: 30 - protein, 11 aa, synthetic construct
  REGION 1..11: note = an artificially synthesized sequence
RASYNIDSYLA

SEQ ID NO: 31 - protein, 16 aa, synthetic construct
  REGION 1..16: note = an artificially synthesized sequence
QPSQEVVHMNRNTYLH

SEQ ID NO: 32 - protein, 16 aa, synthetic construct
  REGION 1..16: note = an artificially synthesized sequence
QPSQEVVHMNRNTYLH

SEQ ID NO: 33 - protein, 7 aa, synthetic construct
  REGION 1..7: note = an artificially synthesized sequence
YSTLLVD

SEQ ID NO: 34 - protein, 7 aa, synthetic construct
  REGION 1..7: note = an artificially synthesized sequence
YSTLLVD

SEQ ID NO: 35 - protein, 7 aa, synthetic construct
  REGION 1..7: note = an artificially synthesized sequence
KVSNRFP

SEQ ID NO: 36 - protein, 7 aa, synthetic construct
  REGION 1..7: note = an artificially synthesized sequence
KVSNRFP

SEQ ID NO: 37 - protein, 9 aa, synthetic construct
  REGION 1..9: note = an artificially synthesized sequence
QHYYSIPYT

SEQ ID NO: 38 - protein, 9 aa, synthetic construct
  REGION 1..9: note = an artificially synthesized sequence
QHYYSIPYT

SEQ ID NO: 39 - protein, 9 aa, synthetic construct
  REGION 1..9: note = an artificially synthesized sequence
AQGTSHPFT

SEQ ID NO: 40 - protein, 9 aa, synthetic construct
  REGION 1..9: note = an artificially synthesized sequence
AQGTSHPFT

SEQ ID NO: 41 - protein, 447 aa, synthetic construct
  REGION 1..447: note = an artificially synthesized sequence
QVQLVESGGGVVQPGGSLRLSCAASGFTFSSYTMSWVREAPGQGLEWMGTISSGGGRTYYPDSVKGRFTISRDNSKNTLYLQMNSLRDEDTAVYYCARGDYRYDGFAYWGEGTLVTVSSASTKGPSVFPLAPSSKSTSGGTAALGCLVEDYFPEPVTVSWNSGALTSGVHTFPAVLESSGLYSLSSVVTVPSSSLGTQTYICNVNHKPSNTKVDERVEPKSCDKTHTCPPCPAPEAAGGPSVFLFPPKPKDTLMISRTPEVTCVVVDVSHEDPEVKFNWYVDGVEVHNAKTKPREEQYASTYRVVSVLTVLHQDWLNGKEYKCKVSNKALPAPIEKTISKAKGQPREPQVYTLPPSREEMTKNQVSLTCLVKGFYPSDIAVEWESNGQPENNYKTTPPVLDSDGSFFLYSKLTVDKSRWQQGNVFSCSVMHEALHNHYTQESLSLSP

SEQ ID NO: 42 - protein, 447 aa, synthetic construct
  REGION 1..447: note = an artificially synthesized sequence
QVQLVESGGGVVQPGGSLRLSCAASGFTFSSYTMSWVRQAPGQGLEWMGTISSGGGRTYYPDSVKGRFTISRDNSKNTLYLQMNSLRDEDTAVYYCARGDYRYDGFAYWGEGTLVTVSSASTKGPSVFPLAPSSKSTSGGTAALGCLVEDYFPEPVTVSWNSGALTSGVHTFPAVLESSGLYSLSSVVTVPSSSLGTQTYICNVNHKPSNTKVDKRVEPKSCDKTHTCPPCPAPEAAGGPSVFLFPPKPKDTLMISRTPEVTCVVVDVSHEDPEVKFNWYVDGVEVHNAKTKPREEQYASTYRVVSVLTVLHQDWLNGKEYKCKVSNKALPAPIEKTISKAKGQPREPQVYTLPPSREEMTKNQVSLTCLVKGFYPSDIAVEWESNGQPENNYKTTPPVLDSDGSFFLYSKLTVDKSRWQQGNVFSCSVMHEALHNHYTQESLSLSP

SEQ ID NO: 43 - protein, 437 aa, synthetic construct
  REGION 1..437: note = an artificially synthesized sequence
DIQMTQSPSSLSASVGDRVTITCRASYNIDSYLAWYQQKPGKAPELLIYYSTLLVDGVPDRFSGSRSGTDFTLTISSLQPEDFATYYCQHYYSIPYTFGQGTKVEIESSASTKGPSVFPLAPSSKSTSGGTAALGCLVKDYFPEPVTVSWNSGALTSGVHTFPAVLQSSGLYSLSSVVTVPSSSLGTQTYICNVNHKPSNTKVDKRVEPKSCDKTHTCPPCPAPEAAGGPSVFLFPPKPKDTLMISRTPEVTCVVVDVSHEDPEVKFNWYVDGVEVHNAKTKPREEQYASTYRVVSVLTVLHQDWLNGKEYKCKVSNKALPAPIEKTISKAKGQPREPQVYTLPPCREEMTKNQVSLWCLVKGFYPSDIAVEWESNGQPENNYKTTPPVLDSDGSFFLYSKLTVDKSRWQEGNVFSCSVMHEALHNHYTQKSLSLSP

SEQ ID NO: 44 - protein, 437 aa, synthetic construct
  REGION 1..437: note = an artificially synthesized sequence
DIQMTQSPSSLSASVGDRVTITCRASYNIDSYLAWYQQKPGKAPELLIYYSTLLVDGVPDRFSGSRSGTDFTLTISSLQPEDFATYYCQHYYSIPYTFGQGTKVEIESSASTKGPSVFPLAPSSKSTSGGTAALGCLVKDYFPEPVTVSWNSGALTSGVHTFPAVLQSSGLYSLSSVVTVPSSSLGTQTYICNVNHKPSNTKVDKRVEPKSCDKTHTCPPCPAPEAAGGPSVFLFPPKPKDTLMISRTPEVTCVVVDVSHEDPEVKFNWYVDGVEVHNAKTKPREEQYASTYRVVSVLTVLHQDWLNGKEYKCKVSNKALPAPIEKTISKAKGQPREPQVYTLPPCREEMTKNQVSLWCLVKGFYPSDIAVEWESNGQPENNYKTTPPVLDSDGSFFLYSKLTVDKSRWQQGNVFSCSVMHEALHNHYTQKSLSLSP

SEQ ID NO: 45 - protein, 447 aa, synthetic construct
  REGION 1..447: note = an artificially synthesized sequence
QVQLVESGGGVVQPGGSLRLSCAASGFTFSSYTMSWVREAPGQGLEWMGTISSGGGRTYYPDSVKGRFTISRDNSKNTLYLQMNSLRDEDTAVYYCARGDYRYDGFAYWGEGTLVTVSSASTKGPSVFPLAPSSKSTSGGTAALGCLVEDYFPEPVTVSWNSGALTSGVHTFPAVLESSGLYSLSSVVTVPSSSLGTQTYICNVNHKPSNTKVDERVEPKSCDKTHTCPPCPAPEAAGGPSVFLFPPKPKDTLMISRTPEVTCVVVDVSHEDPEVKFNWYVDGVEVHNAKTKPREEQYASTYRVVSVLTVLHQDWLNGKEYKCKVSNKALPAPIEKTISKAKGQPREPQVYTLPPSREEMTKNQVSLTCLVKGFYPSDIAVEWESNGQPENNYKTTPPVLDSDGSFFLYSKLTVDKSRWQQGNVFSCSVLHEALHAHYTREELSLSP

SEQ ID NO: 46 - protein, 447 aa, synthetic construct
  REGION 1..447: note = an artificially synthesized sequence
QVQLVESGGGVVQPGGSLRLSCAASGFTFSSYTMSWVRQAPGQGLEWMGTISSGGGRTYYPDSVKGRFTISRDNSKNTLYLQMNSLRDEDTAVYYCARGDYRYDGFAYWGEGTLVTVSSASTKGPSVFPLAPSSKSTSGGTAALGCLVEDYFPEPVTVSWNSGALTSGVHTFPAVLESSGLYSLSSVVTVPSSSLGTQTYICNVNHKPSNTKVDKRVEPKSCDKTHTCPPCPAPEAAGGPSVFLFPPKPKDTLMISRTPEVTCVVVDVSHEDPEVKFNWYVDGVEVHNAKTKPREEQYASTYRVVSVLTVLHQDWLNGKEYKCKVSNKALPAPIEKTISKAKGQPREPQVYTLPPSREEMTKNQVSLTCLVKGFYPSDIAVEWESNGQPENNYKTTPPVLDSDGSFFLYSKLTVDKSRWQQGNVFSCSVLHEALHAHYTREELSLSP

SEQ ID NO: 47 - protein, 437 aa, synthetic construct
  REGION 1..437: note = an artificially synthesized sequence
DIQMTQSPSSLSASVGDRVTITCRASYNIDSYLAWYQQKPGKAPELLIYYSTLLVDGVPDRFSGSRSGTDFTLTISSLQPEDFATYYCQHYYSIPYTFGQGTKVEIESSASTKGPSVFPLAPSSKSTSGGTAALGCLVKDYFPEPVTVSWNSGALTSGVHTFPAVLQSSGLYSLSSVVTVPSSSLGTQTYICNVNHKPSNTKVDKRVEPKSCDKTHTCPPCPAPEAAGGPSVFLFPPKPKDTLMISRTPEVTCVVVDVSHEDPEVKFNWYVDGVEVHNAKTKPREEQYASTYRVVSVLTVLHQDWLNGKEYKCKVSNKALPAPIEKTISKAKGQPREPQVYTLPPCREEMTKNQVSLWCLVKGFYPSDIAVEWESNGQPENNYKTTPPVLDSDGSFFLYSKLTVDKSRWQQGNVFSCSVLHEALHAHYTRKELSLSP

SEQ ID NO: 48 - protein, 447 aa, synthetic construct
  REGION 1..447: note = an artificially synthesized sequence
QVQLVESGGGVVQPGGSLRLSCAASGFTFSSYTMSWVRQAPGQGLEWMGTISSGGGRTYYPDSVKGRFTISRDNSKNTLYLQMNSLRDEDTAVYYCARGDYRYDGFAYWGEGTLVTVSSASTKGPSVFPLAPSSKSTSGGTAALGCLVEDYFPEPVTVSWNSGALTSGVHTFPAVLESSGLYSLSSVVTVPSSSLGTQTYICNVNHKPSNTKVDERVEPKSCDKTHTCPPCPAPEAAGGPSVFLFPPKPKDTLMISRTPEVTCVVVDVSHEDPEVKFNWYVDGVEVHNAKTKPREEQYASTYRVVSVLTVLHQDWLNGKEYKCKVSNKALPAPIEKTISKAKGQPREPQVYTLPPSREEMTKNQVSLTCLVKGFYPSDIAVEWESNGQPENNYKTTPPVLDSDGSFFLYSKLTVDKSRWQQGNVFSCSVMHEALHNHYTQESLSLSP

SEQ ID NO: 49 - protein, 447 aa, synthetic construct
  REGION 1..447: note = an artificially synthesized sequence
QVQLVESGGGVVQPGGSLRLSCAASGFTFSSYTMSWVRQAPGQGLEWMGTISSGGGRTYYPDSVKGRFTISRDNSKNTLYLQMNSLRDEDTAVYYCARGDYRYDGFAYWGEGTLVTVSSASTKGPSVFPLAPSSKSTSGGTAALGCLVEDYFPEPVTVSWNSGALTSGVHTFPAVLESSGLYSLSSVVTVPSSSLGTQTYICNVNHKPSNTKVDERVEPKSCDKTHTCPPCPAPEAAGGPSVFLFPPKPKDTLMISRTPEVTCVVVDVSHEDPEVKFNWYVDGVEVHNAKTKPREEQYASTYRVVSVLTVLHQDWLNGKEYKCKVSNKALPAPIEKTISKAKGQPREPQVYTLPPSREEMTKNQVSLTCLVKGFYPSDIAVEWESNGQPENNYKTTPPVLDSDGSFFLYSKLTVDKSRWQQGNVFSCSVLHEALHAHYTREELSLSP

SEQ ID NO: 50 - protein, 214 aa, synthetic construct
  REGION 1..214: note = an artificially synthesized sequence
DIQMTQSPSSLSASVGDRVTITCRASYNIDSYLAWYQKKPGKAPELLIYYSTLLVDGVPDRFSGSRSGTDFTLTISSLQPEDFATYYCQHYYSIPYTFGQGTKVEIERTVAAPSVFIFPPSDKQLKSGTAKVVCLLNNFYPREAKVQWKVDNALQSGNSKESVTEQDSKDSTYSLSSTLTLSKADYEKHKVYACEVTHQGLSSPVTKSFNRGEC

SEQ ID NO: 51 - protein, 214 aa, synthetic construct
  REGION 1..214: note = an artificially synthesized sequence
DIQMTQSPSSLSASVGDRVTITCRASYNIDSYLAWYQQKPGKAPELLIYYSTLLVDGVPDRFSGSRSGTDFTLTISSLQPEDFATYYCQHYYSIPYTFGQGTKVEIERTVAAPSVFIFPPSDEQLKSGTAKVVCLLNNFYPREAKVQWKVDNALQSGNSKESVTEQDSKDSTYSLSSTLTLSKADYEKHKVYACEVTHQGLSSPVTKSFNRGEC

SEQ ID NO: 52 - protein, 226 aa, synthetic construct
  REGION 1..226: note = an artificially synthesized sequence
QVQLVESGGGVVQPGGSLRLSCAASGFTFSSYTMSWVRQAPGQGLEWMGTISSGGGRTYYPDSVKGRFTISRDNSKNTLYLQMNSLRDEDTAVYYCARGDYRYDGFAYWGEGTLVTVSSASVAAPSVFIFPPSDEQLKSGTASVVCLLNNFYPREAKVQWKVDNALQSGNSQESVTEQDSKDSTYSLSSTLTLSKADYEKHKVYACEVTHQGLSSPVTKSFNRGEC

SEQ ID NO: 53 - protein, 214 aa, synthetic construct
  REGION 1..214: note = an artificially synthesized sequence
DIQMTQSPSSLSASVGDRVTITCRASYNIDSYLAWYQQKPGKAPELLIYYSTLLVDGVPDRFSGSRSGTDFTLTISSLQPEDFATYYCQHYYSIPYTFGQGTKVEIERTVAAPSVFIFPPSDKQLKSGTAKVVCLLNNFYPREAKVQWKVDNALQSGNSKESVTEQDSKDSTYSLSSTLTLSKADYEKHKVYACEVTHQGLSSPVTKSFNRGEC

SEQ ID NO: 54 - protein, 456 aa, synthetic construct
  REGION 1..456: note = an artificially synthesized sequence
QVQLVESGGGLVQPGRSLRLSCAASGFKFSNVWFHWVRKAPGKGLEWVAQIKDYYNAYAAYYAPSVKGRFTISRDDSKNSIYLQMNSLKTEDTAVYYCHYVHYASASTLLPAEGVDAWGQGTTVTVSSASTKGPSVFPLAPSSKSTSGGTAALGCLVKDYFPEPVTVSWNSGALTSGVHTFPAVLKSSGLYSLSSVVTVPSSSLGTQTYICNVNHKPSNTKVDKRVEPKSCDKTHTCPPCPAPEAAGGPSVFLFPPKPKDTLMISRTPEVTCVVVDVSHEDPEVKFNWYVDGVEVHNAKTKPREEQYASTYRVVSVLTVLHQDWLNGKEYKCKVSNKALPAPIEKTISKAKGQPREPQVYTLPPSRKEMTKNQVSLTCLVKGFYPSDIAVEWESNGQPENNYKTTPPVLDSDGSFFLYSKLTVDKSRWQQGNVFSCSVMHEALHNHYTQKSLSLSP

SEQ ID NO: 55 - protein, 456 aa, synthetic construct
  REGION 1..456: note = an artificially synthesized sequence
QVQLVESGGGLVQPGRSLRLSCAASGFKFSNVWFHWVRKAPGKGLEWVAQIKDYYNAYAGYYHPSVKGRFTISRDDSKNSIYLQMNSLKTEDTAVYYCHYVHYAAASQLLPAEGVDAWGQGTTVTVSSASTKGPSVFPLAPSSKSTSGGTAALGCLVKDYFPEPVTVSWNSGALTSGVHTFPAVLKSSGLYSLSSVVTVPSSSLGTQTYICNVNHKPSNTKVDKRVEPKSCDKTHTCPPCPAPEAAGGPSVFLFPPKPKDTLMISRTPEVTCVVVDVSHEDPEVKFNWYVDGVEVHNAKTKPREEQYASTYRVVSVLTVLHQDWLNGKEYKCKVSNKALPAPIEKTISKAKGQPREPQVYTLPPSRKEMTKNQVSLTCLVKGFYPSDIAVEWESNGQPENNYKTTPPVLDSDGSFFLYSKLTVDKSRWQQGNVFSCSVMHEALHNHYTQKSLSLSP

SEQ ID NO: 56 - protein, 456 aa, synthetic construct
  REGION 1..456: note = an artificially synthesized sequence
QVQLVESGGGLVQPGRSLRLSCAASGFKFSNVWFHWVRQAPGKGLEWVAQIKDYYNAYAAYYAPSVKGRFTISRDDSKNSIYLQMNSLKTEDTAVYYCHYVHYASASTLLPAEGVDAWGQGTTVTVSSASTKGPSVFPLAPSSKSTSGGTAALGCLVKDYFPEPVTVSWNSGALTSGVHTFPAVLKSSGLYSLSSVVTVPSSSLGTQTYICNVNHKPSNTKVDKRVEPKSCDKTHTCPPCPAPEAAGGPSVFLFPPKPKDTLMISRTPEVTCVVVDVSHEDPEVKFNWYVDGVEVHNAKTKPREEQYASTYRVVSVLTVLHQDWLNGKEYKCKVSNKALPAPIEKTISKAKGQPREPQVYTLPPSRKEMTKNQVSLTCLVKGFYPSDIAVEWESNGQPENNYKTTPPVLDSDGSFFLYSKLTVDKSRWQQGNVFSCSVMHEALHNHYTQKSLSLSP

SEQ ID NO: 57 - protein, 456 aa, synthetic construct
  REGION 1..456: note = an artificially synthesized sequence
QVQLVESGGGLVQPGRSLRLSCAASGFKFSNVWFHWVRQAPGKGLEWVAQIKDYYNAYAGYYHPSVKGRFTISRDDSKNSIYLQMNSLKTEDTAVYYCHYVHYAAASQLLPAEGVDAWGQGTTVTVSSASTKGPSVFPLAPSSKSTSGGTAALGCLVKDYFPEPVTVSWNSGALTSGVHTFPAVLKSSGLYSLSSVVTVPSSSLGTQTYICNVNHKPSNTKVDKRVEPKSCDKTHTCPPCPAPEAAGGPSVFLFPPKPKDTLMISRTPEVTCVVVDVSHEDPEVKFNWYVDGVEVHNAKTKPREEQYASTYRVVSVLTVLHQDWLNGKEYKCKVSNKALPAPIEKTISKAKGQPREPQVYTLPPSRKEMTKNQVSLTCLVKGFYPSDIAVEWESNGQPENNYKTTPPVLDSDGSFFLYSKLTVDKSRWQQGNVFSCSVMHEALHNHYTQKSLSLSP

SEQ ID NO: 58 - protein, 456 aa, synthetic construct
  REGION 1..456: note = an artificially synthesized sequence
QVQLVESGGGLVQPGRSLRLSCAASGFKFSNVWFHWVRQAPGKGLEWVAQIKDYYNAYAAYYAPSVKGRFTISRDDSKNSIYLQMNSLKTEDTAVYYCHYVHYASASTLLPAEGVDAWGQGTTVTVSSASTKGPSVFPLAPSSKSTSGGTAALGCLVEDYFPEPVTVSWNSGALTSGVHTFPAVLQSSGLYSLSSVVTVPSSSLGTQTYICNVNHKPSNTKVDERVEPKSCDKTHTCPPCPAPEAAGGPSVFLFPPKPKDTLMISRTPEVTCVVVDVSHEDPEVKFNWYVDGVEVHNAKTKPREEQYASTYRVVSVLTVLHQDWLNGKEYKCKVSNKALPAPIEKTISKAKGQPREPQVCTLPPSREEMTKNQVSLSCAVKGFYPSDIAVEWESNGQPENNYKTTPPVLDSDGSFFLVSKLTVDKSRWQEGNVFSCSVMHEALHNHYTQKSLSLSP

SEQ ID NO: 59 - protein, 456 aa, synthetic construct
  REGION 1..456: note = an artificially synthesized sequence
QVQLVESGGGLVQPGRSLRLSCAASGFKFSNVWFHWVRQAPGKGLEWVAQIKDYYNAYAGYYHPSVKGRFTISRDDSKNSIYLQMNSLKTEDTAVYYCHYVHYAAASQLLPAEGVDAWGQGTTVTVSSASTKGPSVFPLAPSSKSTSGGTAALGCLVEDYFPEPVTVSWNSGALTSGVHTFPAVLQSSGLYSLSSVVTVPSSSLGTQTYICNVNHKPSNTKVDERVEPKSCDKTHTCPPCPAPEAAGGPSVFLFPPKPKDTLMISRTPEVTCVVVDVSHEDPEVKFNWYVDGVEVHNAKTKPREEQYASTYRVVSVLTVLHQDWLNGKEYKCKVSNKALPAPIEKTISKAKGQPREPQVCTLPPSREEMTKNQVSLSCAVKGFYPSDIAVEWESNGQPENNYKTTPPVLDSDGSFFLVSKLTVDKSRWQEGNVFSCSVMHEALHNHYTQKSLSLSP

SEQ ID NO: 60 - protein, 456 aa, synthetic construct
  REGION 1..456: note = an artificially synthesized sequence
QVQLVESGGGLVQPGRSLRLSCAASGFKFSNVWFHWVRQAPGKGLEWVAQIKDYYNAYAAYYAPSVKGRFTISRDDSKNSIYLQMNSLKTEDTAVYYCHYVHYASASTLLPAEGVDAWGQGTTVTVSSASTKGPSVFPLAPSSKSTSGGTAALGCLVEDYFPEPVTVSWNSGALTSGVHTFPAVLQSSGLYSLSSVVTVPSSSLGTQTYICNVNHKPSNTKVDERVEPKSCDKTHTCPPCPAPEAAGGPSVFLFPPKPKDTLMISRTPEVTCVVVDVSHEDPEVKFNWYVDGVEVHNAKTKPREEQYASTYRVVSVLTVLHQDWLNGKEYKCKVSNKALPAPIEKTISKAKGQPREPQVCTLPPSREEMTKNQVSLSCAVKGFYPSDIAVEWESNGQPENNYKTTPPVLDSDGSFFLVSKLTVDKSRWQQGNVFSCSVMHEALHNHYTQKSLSLSP

SEQ ID NO: 61 - protein, 456 aa, synthetic construct
  REGION 1..456: note = an artificially synthesized sequence
QVQLVESGGGLVQPGRSLRLSCAASGFKFSNVWFHWVRQAPGKGLEWVAQIKDYYNAYAGYYHPSVKGRFTISRDDSKNSIYLQMNSLKTEDTAVYYCHYVHYAAASQLLPAEGVDAWGQGTTVTVSSASTKGPSVFPLAPSSKSTSGGTAALGCLVEDYFPEPVTVSWNSGALTSGVHTFPAVLQSSGLYSLSSVVTVPSSSLGTQTYICNVNHKPSNTKVDERVEPKSCDKTHTCPPCPAPEAAGGPSVFLFPPKPKDTLMISRTPEVTCVVVDVSHEDPEVKFNWYVDGVEVHNAKTKPREEQYASTYRVVSVLTVLHQDWLNGKEYKCKVSNKALPAPIEKTISKAKGQPREPQVCTLPPSREEMTKNQVSLSCAVKGFYPSDIAVEWESNGQPENNYKTTPPVLDSDGSFFLVSKLTVDKSRWQQGNVFSCSVMHEALHNHYTQKSLSLSP

SEQ ID NO: 62 - protein, 456 aa, synthetic construct
  REGION 1..456: note = an artificially synthesized sequence
QVQLVESGGGLVQPGRSLRLSCAASGFKFSNVWFHWVRKAPGKGLEWVAQIKDYYNAYAAYYAPSVKGRFTISRDDSKNSIYLQMNSLKTEDTAVYYCHYVHYASASTLLPAEGVDAWGQGTTVTVSSASTKGPSVFPLAPSSKSTSGGTAALGCLVKDYFPEPVTVSWNSGALTSGVHTFPAVLKSSGLYSLSSVVTVPSSSLGTQTYICNVNHKPSNTKVDKRVEPKSCDKTHTCPPCPAPEAAGGPSVFLFPPKPKDTLMISRTPEVTCVVVDVSHEDPEVKFNWYVDGVEVHNAKTKPREEQYASTYRVVSVLTVLHQDWLNGKEYKCKVSNKALPAPIEKTISKAKGQPREPQVYTLPPSRKEMTKNQVSLTCLVKGFYPSDIAVEWESNGQPENNYKTTPPVLDSDGSFFLYSKLTVDKSRWQQGNVFSCSVLHEALHAHYTRKELSLSP

SEQ ID NO: 63 - protein, 456 aa, synthetic construct
  REGION 1..456: note = an artificially synthesized sequence
QVQLVESGGGLVQPGRSLRLSCAASGFKFSNVWFHWVRKAPGKGLEWVAQIKDYYNAYAGYYHPSVKGRFTISRDDSKNSIYLQMNSLKTEDTAVYYCHYVHYAAASQLLPAEGVDAWGQGTTVTVSSASTKGPSVFPLAPSSKSTSGGTAALGCLVKDYFPEPVTVSWNSGALTSGVHTFPAVLKSSGLYSLSSVVTVPSSSLGTQTYICNVNHKPSNTKVDKRVEPKSCDKTHTCPPCPAPEAAGGPSVFLFPPKPKDTLMISRTPEVTCVVVDVSHEDPEVKFNWYVDGVEVHNAKTKPREEQYASTYRVVSVLTVLHQDWLNGKEYKCKVSNKALPAPIEKTISKAKGQPREPQVYTLPPSRKEMTKNQVSLTCLVKGFYPSDIAVEWESNGQPENNYKTTPPVLDSDGSFFLYSKLTVDKSRWQQGNVFSCSVLHEALHAHYTRKELSLSP

SEQ ID NO: 64 - protein, 456 aa, synthetic construct
  REGION 1..456: note = an artificially synthesized sequence
QVQLVESGGGLVQPGRSLRLSCAASGFKFSNVWFHWVRQAPGKGLEWVAQIKDYYNAYAAYYAPSVKGRFTISRDDSKNSIYLQMNSLKTEDTAVYYCHYVHYASASTLLPAEGVDAWGQGTTVTVSSASTKGPSVFPLAPSSKSTSGGTAALGCLVKDYFPEPVTVSWNSGALTSGVHTFPAVLKSSGLYSLSSVVTVPSSSLGTQTYICNVNHKPSNTKVDKRVEPKSCDKTHTCPPCPAPEAAGGPSVFLFPPKPKDTLMISRTPEVTCVVVDVSHEDPEVKFNWYVDGVEVHNAKTKPREEQYASTYRVVSVLTVLHQDWLNGKEYKCKVSNKALPAPIEKTISKAKGQPREPQVYTLPPSRKEMTKNQVSLTCLVKGFYPSDIAVEWESNGQPENNYKTTPPVLDSDGSFFLYSKLTVDKSRWQQGNVFSCSVLHEALHAHYTRKELSLSP

SEQ ID NO: 65 - protein, 456 aa, synthetic construct
  REGION 1..456: note = an artificially synthesized sequence
QVQLVESGGGLVQPGRSLRLSCAASGFKFSNVWFHWVRQAPGKGLEWVAQIKDYYNAYAGYYHPSVKGRFTISRDDSKNSIYLQMNSLKTEDTAVYYCHYVHYAAASQLLPAEGVDAWGQGTTVTVSSASTKGPSVFPLAPSSKSTSGGTAALGCLVKDYFPEPVTVSWNSGALTSGVHTFPAVLKSSGLYSLSSVVTVPSSSLGTQTYICNVNHKPSNTKVDKRVEPKSCDKTHTCPPCPAPEAAGGPSVFLFPPKPKDTLMISRTPEVTCVVVDVSHEDPEVKFNWYVDGVEVHNAKTKPREEQYASTYRVVSVLTVLHQDWLNGKEYKCKVSNKALPAPIEKTISKAKGQPREPQVYTLPPSRKEMTKNQVSLTCLVKGFYPSDIAVEWESNGQPENNYKTTPPVLDSDGSFFLYSKLTVDKSRWQQGNVFSCSVLHEALHAHYTRKELSLSP

SEQ ID NO: 66 - protein, 456 aa, synthetic construct
  REGION 1..456: note = an artificially synthesized sequence
QVQLVESGGGLVQPGRSLRLSCAASGFKFSNVWFHWVRQAPGKGLEWVAQIKDYYNAYAAYYAPSVKGRFTISRDDSKNSIYLQMNSLKTEDTAVYYCHYVHYASASTLLPAEGVDAWGQGTTVTVSSASTKGPSVFPLAPSSKSTSGGTAALGCLVEDYFPEPVTVSWNSGALTSGVHTFPAVLQSSGLYSLSSVVTVPSSSLGTQTYICNVNHKPSNTKVDERVEPKSCDKTHTCPPCPAPEAAGGPSVFLFPPKPKDTLMISRTPEVTCVVVDVSHEDPEVKFNWYVDGVEVHNAKTKPREEQYASTYRVVSVLTVLHQDWLNGKEYKCKVSNKALPAPIEKTISKAKGQPREPQVCTLPPSREEMTKNQVSLSCAVKGFYPSDIAVEWESNGQPENNYKTTPPVLDSDGSFFLVSKLTVDKSRWQQGNVFSCSVLHEALHAHYTRKELSLSP

SEQ ID NO: 67 - protein, 456 aa, synthetic construct
  REGION 1..456: note = an artificially synthesized sequence
QVQLVESGGGLVQPGRSLRLSCAASGFKFSNVWFHWVRQAPGKGLEWVAQIKDYYNAYAGYYHPSVKGRFTISRDDSKNSIYLQMNSLKTEDTAVYYCHYVHYAAASQLLPAEGVDAWGQGTTVTVSSASTKGPSVFPLAPSSKSTSGGTAALGCLVEDYFPEPVTVSWNSGALTSGVHTFPAVLQSSGLYSLSSVVTVPSSSLGTQTYICNVNHKPSNTKVDERVEPKSCDKTHTCPPCPAPEAAGGPSVFLFPPKPKDTLMISRTPEVTCVVVDVSHEDPEVKFNWYVDGVEVHNAKTKPREEQYASTYRVVSVLTVLHQDWLNGKEYKCKVSNKALPAPIEKTISKAKGQPREPQVCTLPPSREEMTKNQVSLSCAVKGFYPSDIAVEWESNGQPENNYKTTPPVLDSDGSFFLVSKLTVDKSRWQQGNVFSCSVLHEALHAHYTRKELSLSP

SEQ ID NO: 68 - protein, 219 aa, synthetic construct
  REGION 1..219: note = an artificially synthesized sequence
DIVMTQSPLSLPVTPGEPASISCQPSQEVVHMNRNTYLHWYQEKPGQAPRLLIYKVSNRFPGVPDRFSGSGSGTDFTLKISRVEAEDVGVYYCAQGTSHPFTFGQGTKLEIKRTVAAPSVFIFPPSDEQLKSGTAEVVCLLNNFYPREAKVQWKVDNALQSGNSEESVTEQDSKDSTYSLSSTLELSKADYEKHKVYACEVTHQGLSSPVTKSFNRGEC

SEQ ID NO: 69 - protein, 219 aa, synthetic construct
  REGION 1..219: note = an artificially synthesized sequence
DIVMTQSPLSLPVTPGEPASISCQPSQEVVHMNRNTYLHWYQQKPGQAPRLLIYKVSNRFPGVPDRFSGSGSGTDFTLKISRVEAEDVGVYYCAQGTSHPFTFGQGTKLEIKRTVAAPSVFIFPPSDEQLKSGTAEVVCLLNNFYPREAKVQWKVDNALQSGNSEESVTEQDSKDSTYSLSSTLTLSKADYEKHKVYACEVTHQGLSSPVTKSFNRGEC

SEQ ID NO: 70 - protein, 219 aa, synthetic construct
  REGION 1..219: note = an artificially synthesized sequence
DIVMTQSPLSLPVTPGEPASISCQPSQEVVHMNRNTYLHWYQQKPGQAPRLLIYKVSNRFPGVPDRFSGSGSGTDFTLKISRVEAEDVGVYYCAQGTSHPFTFGQGTKLEIKRTVAAPSVFIFPPSDRKLKSGTASVVCLLNNFYPREAKVQWKVDNALQSGNSQESVTEQDSKDSTYSLSSTLTLSKADYEKHKVYACEVTHQGLSSPVTKSFNRGEC

SEQ ID NO: 71 - protein, 219 aa, synthetic construct
  REGION 1..219: note = an artificially synthesized sequence
DIVMTQSPLSLPVTPGEPASISCQPSQEVVHMNRNTYLHWYQQKPGQAPRLLIYKVSNRFPGVPDRFSGSGSGTDFTLKISRVEAEDVGVYYCAQGTSHPFTFGQGTKLEIKRTVAAPSVFIFPPSDEQLKSGTAEVVCLLNNFYPREAKVQWKVDNALQSGNSEESVTEQDSKDSTYSLSSTLELSKADYEKHKVYACEVTHQGLSSPVTKSFNRGEC

SEQ ID NO: 72 - protein, 107 aa, synthetic construct
  REGION 1..107: note = an artificially synthesized sequence
RTVAAPSVFIFPPSDRKLKSGTASVVCLLNNFYPREAKVQWKVDNALQSGNSQESVTEQDSKDSTYSLSSTLTLSKADYEKHKVYACEVTHQGLSSPVTKSFNRGEC

SEQ ID NO: 73 - protein, 328 aa, synthetic construct
  REGION 1..328: note = an artificially synthesized sequence
ASTKGPSVFPLAPSSKSTSGGTAALGCLVEDYFPEPVTVSWNSGALTSGVHTFPAVLESSGLYSLSSVVTVPSSSLGTQTYICNVNHKPSNTKVDERVEPKSCDKTHTCPPCPAPEAAGGPSVFLFPPKPKDTLMISRTPEVTCVVVDVSHEDPEVKFNWYVDGVEVHNAKTKPREEQYASTYRVVSVLTVLHQDWLNGKEYKCKVSNKALPAPIEKTISKAKGQPREPQVYTLPPSREEMTKNQVSLTCLVKGFYPSDIAVEWESNGQPENNYKTTPPVLDSDGSFFLYSKLTVDKSRWQQGNVFSCSVMHEALHNHYTQESLSLSP

SEQ ID NO: 74 - protein, 328 aa, synthetic construct
  REGION 1..328: note = an artificially synthesized sequence
ASTKGPSVFPLAPSSKSTSGGTAALGCLVKDYFPEPVTVSWNSGALTSGVHTFPAVLKSSGLYSLSSVVTVPSSSLGTQTYICNVNHKPSNTKVDKRVEPKSCDKTHTCPPCPAPEAAGGPSVFLFPPKPKDTLMISRTPEVTCVVVDVSHEDPEVKFNWYVDGVEVHNAKTKPREEQYASTYRVVSVLTVLHQDWLNGKEYKCKVSNKALPAPIEKTISKAKGQPREPQVYTLPPSRKEMTKNQVSLTCLVKGFYPSDIAVEWESNGQPENNYKTTPPVLDSDGSFFLYSKLTVDKSRWQQGNVFSCSVMHEALHNHYTQKSLSLSP

SEQ ID NO: 75 - protein, 328 aa, synthetic construct
  REGION 1..328: note = an artificially synthesized sequence
ASTKGPSVFPLAPSSKSTSGGTAALGCLVEDYFPEPVTVSWNSGALTSGVHTFPAVLQSSGLYSLSSVVTVPSSSLGTQTYICNVNHKPSNTKVDERVEPKSCDKTHTCPPCPAPEAAGGPSVFLFPPKPKDTLMISRTPEVTCVVVDVSHEDPEVKFNWYVDGVEVHNAKTKPREEQYASTYRVVSVLTVLHQDWLNGKEYKCKVSNKALPAPIEKTISKAKGQPREPQVCTLPPSREEMTKNQVSLSCAVKGFYPSDIAVEWESNGQPENNYKTTPPVLDSDGSFFLVSKLTVDKSRWQEGNVFSCSVMHEALHNHYTQKSLSLSP

SEQ ID NO: 76 - protein, 330 aa, synthetic construct
  REGION 1..330: note = an artificially synthesized sequence
SSASTKGPSVFPLAPSSKSTSGGTAALGCLVKDYFPEPVTVSWNSGALTSGVHTFPAVLQSSGLYSLSSVVTVPSSSLGTQTYICNVNHKPSNTKVDKRVEPKSCDKTHTCPPCPAPEAAGGPSVFLFPPKPKDTLMISRTPEVTCVVVDVSHEDPEVKFNWYVDGVEVHNAKTKPREEQYASTYRVVSVLTVLHQDWLNGKEYKCKVSNKALPAPIEKTISKAKGQPREPQVYTLPPCREEMTKNQVSLWCLVKGFYPSDIAVEWESNGQPENNYKTTPPVLDSDGSFFLYSKLTVDKSRWQEGNVFSCSVMHEALHNHYTQKSLSLSP

SEQ ID NO: 77 - protein, 328 aa, synthetic construct
  REGION 1..328: note = an artificially synthesized sequence
ASTKGPSVFPLAPSSKSTSGGTAALGCLVEDYFPEPVTVSWNSGALTSGVHTFPAVLQSSGLYSLSSVVTVPSSSLGTQTYICNVNHKPSNTKVDERVEPKSCDKTHTCPPCPAPEAAGGPSVFLFPPKPKDTLMISRTPEVTCVVVDVSHEDPEVKFNWYVDGVEVHNAKTKPREEQYASTYRVVSVLTVLHQDWLNGKEYKCKVSNKALPAPIEKTISKAKGQPREPQVCTLPPSREEMTKNQVSLSCAVKGFYPSDIAVEWESNGQPENNYKTTPPVLDSDGSFFLVSKLTVDKSRWQQGNVFSCSVLHEALHAHYTRKELSLSP

SEQ ID NO: 78 - protein, 330 aa, synthetic construct
  REGION 1..330: note = an artificially synthesized sequence
SSASTKGPSVFPLAPSSKSTSGGTAALGCLVKDYFPEPVTVSWNSGALTSGVHTFPAVLQSSGLYSLSSVVTVPSSSLGTQTYICNVNHKPSNTKVDKRVEPKSCDKTHTCPPCPAPEAAGGPSVFLFPPKPKDTLMISRTPEVTCVVVDVSHEDPEVKFNWYVDGVEVHNAKTKPREEQYASTYRVVSVLTVLHQDWLNGKEYKCKVSNKALPAPIEKTISKAKGQPREPQVYTLPPCREEMTKNQVSLWCLVKGFYPSDIAVEWESNGQPENNYKTTPPVLDSDGSFFLYSKLTVDKSRWQQGNVFSCSVLHEALHAHYTRKELSLSP

SEQ ID NO: 79 - protein, 328 aa, synthetic construct
  REGION 1..328: note = an artificially synthesized sequence
ASTKGPSVFPLAPSSKSTSGGTAALGCLVEDYFPEPVTVSWNSGALTSGVHTFPAVLQSSGLYSLSSVVTVPSSSLGTQTYICNVNHKPSNTKVDERVEPKSCDKTHTCPPCPAPEAAGGPSVFLFPPKPKDTLMISRTPEVTCVVVDVSHEDPEVKFNWYVDGVEVHNAKTKPREEQYASTYRVVSVLTVLHQDWLNGKEYKCKVSNKALPAPIEKTISKAKGQPREPQVCTLPPSREEMTKNQVSLSCAVKGFYPSDIAVEWESNGQPENNYKTTPPVLDSDGSFFLVSKLTVDKSRWQQGNVFSCSVMHEALHNHYTQKSLSLSP

SEQ ID NO: 80 - protein, 330 aa, synthetic construct
  REGION 1..330: note = an artificially synthesized sequence
SSASTKGPSVFPLAPSSKSTSGGTAALGCLVKDYFPEPVTVSWNSGALTSGVHTFPAVLQSSGLYSLSSVVTVPSSSLGTQTYICNVNHKPSNTKVDKRVEPKSCDKTHTCPPCPAPEAAGGPSVFLFPPKPKDTLMISRTPEVTCVVVDVSHEDPEVKFNWYVDGVEVHNAKTKPREEQYASTYRVVSVLTVLHQDWLNGKEYKCKVSNKALPAPIEKTISKAKGQPREPQVYTLPPCREEMTKNQVSLWCLVKGFYPSDIAVEWESNGQPENNYKTTPPVLDSDGSFFLYSKLTVDKSRWQQGNVFSCSVMHEALHNHYTQKSLSLSP

SEQ ID NO: 81 - protein, 328 aa, synthetic construct
  REGION 1..328: note = an artificially synthesized sequence
ASTKGPSVFPLAPSSKSTSGGTAALGCLVEDYFPEPVTVSWNSGALTSGVHTFPAVLESSGLYSLSSVVTVPSSSLGTQTYICNVNHKPSNTKVDKRVEPKSCDKTHTCPPCPAPEAAGGPSVFLFPPKPKDTLMISRTPEVTCVVVDVSHEDPEVKFNWYVDGVEVHNAKTKPREEQYASTYRVVSVLTVLHQDWLNGKEYKCKVSNKALPAPIEKTISKAKGQPREPQVYTLPPSREEMTKNQVSLTCLVKGFYPSDIAVEWESNGQPENNYKTTPPVLDSDGSFFLYSKLTVDKSRWQQGNVFSCSVMHEALHNHYTQESLSLSP

SEQ ID NO: 82 - protein, 328 aa, synthetic construct
  REGION 1..328: note = an artificially synthesized sequence
ASTKGPSVFPLAPSSKSTSGGTAALGCLVEDYFPEPVTVSWNSGALTSGVHTFPAVLESSGLYSLSSVVTVPSSSLGTQTYICNVNHKPSNTKVDERVEPKSCDKTHTCPPCPAPEAAGGPSVFLFPPKPKDTLMISRTPEVTCVVVDVSHEDPEVKFNWYVDGVEVHNAKTKPREEQYASTYRVVSVLTVLHQDWLNGKEYKCKVSNKALPAPIEKTISKAKGQPREPQVYTLPPSREEMTKNQVSLTCLVKGFYPSDIAVEWESNGQPENNYKTTPPVLDSDGSFFLYSKLTVDKSRWQQGNVFSCSVLHEALHAHYTREELSLSP

SEQ ID NO: 83 - protein, 328 aa, synthetic construct
  REGION 1..328: note = an artificially synthesized sequence
ASTKGPSVFPLAPSSKSTSGGTAALGCLVKDYFPEPVTVSWNSGALTSGVHTFPAVLKSSGLYSLSSVVTVPSSSLGTQTYICNVNHKPSNTKVDKRVEPKSCDKTHTCPPCPAPEAAGGPSVFLFPPKPKDTLMISRTPEVTCVVVDVSHEDPEVKFNWYVDGVEVHNAKTKPREEQYASTYRVVSVLTVLHQDWLNGKEYKCKVSNKALPAPIEKTISKAKGQPREPQVYTLPPSRKEMTKNQVSLTCLVKGFYPSDIAVEWESNGQPENNYKTTPPVLDSDGSFFLYSKLTVDKSRWQQGNVFSCSVLHEALHAHYTRKELSLSP

SEQ ID NO: 84 - protein, 328 aa, synthetic construct
  REGION 1..328: note = an artificially synthesized sequence
ASTKGPSVFPLAPSSKSTSGGTAALGCLVEDYFPEPVTVSWNSGALTSGVHTFPAVLESSGLYSLSSVVTVPSSSLGTQTYICNVNHKPSNTKVDKRVEPKSCDKTHTCPPCPAPEAAGGPSVFLFPPKPKDTLMISRTPEVTCVVVDVSHEDPEVKFNWYVDGVEVHNAKTKPREEQYASTYRVVSVLTVLHQDWLNGKEYKCKVSNKALPAPIEKTISKAKGQPREPQVYTLPPSREEMTKNQVSLTCLVKGFYPSDIAVEWESNGQPENNYKTTPPVLDSDGSFFLYSKLTVDKSRWQQGNVFSCSVLHEALHAHYTREELSLSP

SEQ ID NO: 85 - protein, 107 aa, synthetic construct
  REGION 1..107: note = an artificially synthesized sequence
RTVAAPSVFIFPPSDEQLKSGTAEVVCLLNNFYPREAKVQWKVDNALQSGNSEESVTEQDSKDSTYSLSSTLTLSKADYEKHKVYACEVTHQGLSSPVTKSFNRGEC

SEQ ID NO: 86 - protein, 107 aa, synthetic construct
  REGION 1..107: note = an artificially synthesized sequence
RTVAAPSVFIFPPSDEQLKSGTAKVVCLLNNFYPREAKVQWKVDNALQSGNSKESVTEQDSKDSTYSLSSTLTLSKADYEKHKVYACEVTHQGLSSPVTKSFNRGEC

SEQ ID NO: 87 - protein, 107 aa, synthetic construct
  REGION 1..107: note = an artificially synthesized sequence
RTVAAPSVFIFPPSDEQLKSGTAEVVCLLNNFYPREAKVQWKVDNALQSGNSEESVTEQDSKDSTYSLSSTLELSKADYEKHKVYACEVTHQGLSSPVTKSFNRGEC

SEQ ID NO: 88 - protein, 107 aa, synthetic construct
  REGION 1..107: note = an artificially synthesized sequence
RTVAAPSVFIFPPSDKQLKSGTAKVVCLLNNFYPREAKVQWKVDNALQSGNSKESVTEQDSKDSTYSLSSTLTLSKADYEKHKVYACEVTHQGLSSPVTKSFNRGEC

SEQ ID NO: 89 - protein, 107 aa, synthetic construct
  REGION 1..107: note = an artificially synthesized sequence
ASVAAPSVFIFPPSDEQLKSGTASVVCLLNNFYPREAKVQWKVDNALQSGNSQESVTEQDSKDSTYSLSSTLTLSKADYEKHKVYACEVTHQGLSSPVTKSFNRGEC

SEQ ID NO: 90 - protein, 128 aa, synthetic construct
  REGION 1..128: note = an artificially synthesized sequence
QVQLVESGGGLVQPGRSLRLSCAASGFTFSNAWMHWVRQAPGKGLEWVAQIKDKGNAYAAYYAPSVKGRFTISRDDSKNSIYLQMNSLKTEDTAVYYCHYVHYASASTVLPAFGVDAWGQGTTVTVSS

SEQ ID NO: 91 - protein, 128 aa, synthetic construct
  REGION 1..128: note = an artificially synthesized sequence
QVQLVESGGGLVQPGRSLRLSCAASGFKFSNVWMHWVRQAPGKGLEWVAQIKDKYNAYAAYYAPSVKGRFTISRDDSKNSIYLQMNSLKTEDTAVYYCHYVHYASASTLLPAFGVDAWGQGTTVTVSS

SEQ ID NO: 92 - protein, 128 aa, synthetic construct
  REGION 1..128: note = an artificially synthesized sequence
QVQLVESGGGLVQPGRSLRLSCAASGFKFSNVWMHWVRQAPGKGLEWVAQIKDKYNAYAAYYAPSVKGRFTISRDDSKNSIYLQMNSLKTEDTAVYYCHYIHYASASTLLPAFGVDAWGQGTTVTVSS

SEQ ID NO: 93 - protein, 128 aa, synthetic construct
  REGION 1..128: note = an artificially synthesized sequence
QVQLVESGGGLVQPGRSLRLSCAASGFKFSNVWFHWVRQAPGKGLEWVAQIKDKYNAYATYYAPSVKGRFTISRDDSKNSIYLQMNSLKTEDTAVYYCHYVHYASASTLLPAFGVDAWGQGTTVTVSS

SEQ ID NO: 94 - protein, 128 aa, synthetic construct
  REGION 1..128: note = an artificially synthesized sequence
QVQLVESGGGLVQPGRSLRLSCAASGFVFSNVWMHWVRQAPGKGLEWVAQIKDKWNAYAAYYAPSVKGRFTISRDDSKNSIYLQMNSLKTEDTAVYYCHYIHYASASTLLPAEGIDAWGQGTTVTVSS

SEQ ID NO: 95 - protein, 128 aa, synthetic construct; identical to SEQ ID NO: 5
  REGION 1..128: note = an artificially synthesized sequence

SEQ ID NO: 96 - protein, 128 aa, synthetic construct
  REGION 1..128: note = an artificially synthesized sequence
QVQLVESGGGLVQPGRSLRLSCAASGFKFSNTWFHWVRQAPGKGLEWVAQIKDYYNDYAAYYAPSVKGRFTISRDDSKNSIYLQMNSLKTEDTAVYYCHYVHYASASTLLPAEGVDAWGQGTTVTVSS

SEQ ID NO: 97 - protein, 128 aa, synthetic construct
  REGION 1..128: note = an artificially synthesized sequence
QVQLVESGGGLVQPGRSLRLSCAASGFVFSNVWFHWVRQAPGKGLEWVAQIKDKYNAYADYYAPSVKERFTISRDDSKNSIYLQMNSLKTEDTAVYYCHYVHYASASTLLPAEGVDAWGQGTTVTVSS

SEQ ID NO: 98 - protein, 128 aa, synthetic construct
  REGION 1..128: note = an artificially synthesized sequence
QVQLVESGGGLVQPGRSLRLSCAASGFVFSNVWFHWVRQAPGKGLEWVAQIKDKYNAYADYYAPSVEGRFTISRDDSKNSIYLQMNSLKTEDTAVYYCHYVHYASASTLLPAEGVDAWGQGTTVTVSS

SEQ ID NO: 99 - protein, 128 aa, synthetic construct
  REGION 1..128: note = an artificially synthesized sequence
QVQLVESGGGLVQPGRSLRLSCAASGFVFSNVWFHWVRQAPGKGLEWVAQIKDYYNAYADYYAPSVEGRFTISRDDSKNSIYLQMNSLKTEDTAVYYCHYVHYASASTLLPAEGVDAWGQGTTVTVSS

SEQ ID NO: 100 - protein, 128 aa, synthetic construct
  REGION 1..128: note = an artificially synthesized sequence
QVQLVESGGGLVQPGRSLRLSCAASGFVFSNVWFHWVRQAPGKGLEWVAQIKDKWNAYADYYAPSVKERFTISRDDSKNSIYLQMNSLKTEDTAVYYCHYIHYASASTLLPAEGIDAWGQGTTVTVSS

SEQ ID NO: 101 - protein, 128 aa, synthetic construct
  REGION 1..128: note = an artificially synthesized sequence
QVQLVESGGGLVQPGRSLRLSCAASGFKFSNVWFHWVRQAPGKGLEWVAQIKDYYNAYAGYYHPSVKGRFTISRDDSKNSIYLQMNSLKTEDTAVYYCHYVHYAAASTLLPAEGVDAWGQGTTVTVSS

SEQ ID NO: 102 - protein, 128 aa, synthetic construct; identical to SEQ ID NO: 6
  REGION 1..128: note = an artificially synthesized sequence

SEQ ID NO: 103 - protein, 5 aa, synthetic construct
  REGION 1..5: note = an artificially synthesized sequence
NAWMH

SEQ ID NO: 104 - protein, 5 aa, synthetic construct
  REGION 1..5: note = an artificially synthesized sequence
NVWMH

SEQ ID NO: 105 - protein, 5 aa, synthetic construct
  REGION 1..5: note = an artificially synthesized sequence
NVWMH

SEQ ID NO: 106 - protein, 5 aa, synthetic construct
  REGION 1..5: note = an artificially synthesized sequence
NVWFH

SEQ ID NO: 107 - protein, 5 aa, synthetic construct
  REGION 1..5: note = an artificially synthesized sequence
NVWMH

SEQ ID NO: 108 - protein, 5 aa, synthetic construct
  REGION 1..5: note = an artificially synthesized sequence
NVWFH

SEQ ID NO: 109 - protein, 5 aa, synthetic construct
  REGION 1..5: note = an artificially synthesized sequence
NTWFH

SEQ ID NO: 110 - protein, 5 aa, synthetic construct
  REGION 1..5: note = an artificially synthesized sequence
NVWFH

SEQ ID NO: 111 - protein, 5 aa, synthetic construct
  REGION 1..5: note = an artificially synthesized sequence
NVWFH

SEQ ID NO: 112 - protein, 5 aa, synthetic construct
  REGION 1..5: note = an artificially synthesized sequence
NVWFH

SEQ ID NO: 113 - protein, 5 aa, synthetic construct
  REGION 1..5: note = an artificially synthesized sequence
NVWFH

SEQ ID NO: 114 - protein, 5 aa, synthetic construct
  REGION 1..5: note = an artificially synthesized sequence
NVWFH

SEQ ID NO: 115 - protein, 5 aa, synthetic construct
  REGION 1..5: note = an artificially synthesized sequence
NVWFH

SEQ ID NO: 116 - protein, 19 aa, synthetic construct
  REGION 1..19: note = an artificially synthesized sequence
QIKDKGNAYAAYYAPSVKG

SEQ ID NO: 117 - protein, 19 aa, synthetic construct
  REGION 1..19: note = an artificially synthesized sequence
QIKDKYNAYAAYYAPSVKG

SEQ ID NO: 118 - protein, 19 aa, synthetic construct
  REGION 1..19: note = an artificially synthesized sequence
QIKDKYNAYAAYYAPSVKG

SEQ ID NO: 119 - protein, 19 aa, synthetic construct
  REGION 1..19: note = an artificially synthesized sequence
QIKDKYNAYATYYAPSVKG

SEQ ID NO: 120 - protein, 19 aa, synthetic construct
  REGION 1..19: note = an artificially synthesized sequence
QIKDKWNAYAAYYAPSVKG

SEQ ID NO: 121 - protein, 19 aa, synthetic construct
  REGION 1..19: note = an artificially synthesized sequence
QIKDYYNAYAAYYAPSVKG

SEQ ID NO: 122 - protein, 19 aa, synthetic construct
  REGION 1..19: note = an artificially synthesized sequence
QIKDYYNDYAAYYAPSVKG

SEQ ID NO: 123 - protein, 19 aa, synthetic construct
  REGION 1..19: note = an artificially synthesized sequence
QIKDKYNAYADYYAPSVKE

SEQ ID NO: 124 - protein, 19 aa, synthetic construct
  REGION 1..19: note = an artificially synthesized sequence
QIKDKYNAYADYYAPSVEG

SEQ ID NO: 125 - protein, 19 aa, synthetic construct
  REGION 1..19: note = an artificially synthesized sequence
QIKDYYNAYADYYAPSVEG

SEQ ID NO: 126 - protein, 19 aa, synthetic construct
  REGION 1..19: note = an artificially synthesized sequence
QIKDKWNAYADYYAPSVKE

SEQ ID NO: 127 - protein, 19 aa, synthetic construct
  REGION 1..19: note = an artificially synthesized sequence
QIKDYYNAYAGYYHPSVKG

SEQ ID NO: 128 - protein, 19 aa, synthetic construct
  REGION 1..19: note = an artificially synthesized sequence
QIKDYYNAYAGYYHPSVKG

SEQ ID NO: 129 - protein, 17 aa, synthetic construct
  REGION 1..17: note = an artificially synthesized sequence
VHYASASTVLPAFGVDA

SEQ ID NO: 130 - protein, 17 aa, synthetic construct
  REGION 1..17: note = an artificially synthesized sequence
VHYASASTLLPAFGVDA

SEQ ID NO: 131 - protein, 17 aa, synthetic construct
  REGION 1..17: note = an artificially synthesized sequence
IHYASASTLLPAFGVDA

SEQ ID NO: 132 - protein, 17 aa, synthetic construct
  REGION 1..17: note = an artificially synthesized sequence
VHYASASTLLPAFGVDA

SEQ ID NO: 133 - protein, 17 aa, synthetic construct
  REGION 1..17: note = an artificially synthesized sequence
IHYASASTLLPAEGIDA

SEQ ID NO: 134 - protein, 17 aa, synthetic construct
  REGION 1..17: note = an artificially synthesized sequence
VHYASASTLLPAEGVDA

SEQ ID NO: 135 - protein, 17 aa, synthetic construct
  REGION 1..17: note = an artificially synthesized sequence
VHYASASTLLPAEGVDA

SEQ ID NO: 136 - protein, 17 aa, synthetic construct
  REGION 1..17: note = an artificially synthesized sequence
VHYASASTLLPAEGVDA

SEQ ID NO: 137 - protein, 17 aa, synthetic construct
  REGION 1..17: note = an artificially synthesized sequence
VHYASASTLLPAEGVDA

SEQ ID NO: 138 - protein, 17 aa, synthetic construct
  REGION 1..17: note = an artificially synthesized sequence
VHYASASTLLPAEGVDA

SEQ ID NO: 139 - protein, 17 aa, synthetic construct
  REGION 1..17: note = an artificially synthesized sequence
IHYASASTLLPAEGIDA

SEQ ID NO: 140 - protein, 17 aa, synthetic construct
  REGION 1..17: note = an artificially synthesized sequence
VHYAAASTLLPAEGVDA

SEQ ID NO: 141 - protein, 17 aa, synthetic construct
  REGION 1..17: note = an artificially synthesized sequence
VHYAAASQLLPAEGVDA

SEQ ID NO: 142 - protein, 112 aa, synthetic construct
  REGION 1..112: note = an artificially synthesized sequence
DIVMTQSPLSLPVTPGEPASISCQASQELVHMNRNTYLHWYQQKPGQAPRLLIYKVSNRFPGVPDRFSGSGSGTDFTLKISRVEAEDVGVYYCAQGTSVPFTFGQGTKLEIK

SEQ ID NO: 143 - protein, 112 aa, synthetic construct; identical to SEQ ID NO: 28
  REGION 1..112: note = an artificially synthesized sequence

SEQ ID NO: 144 - protein, 112 aa, synthetic construct
  REGION 1..112: note = an artificially synthesized sequence
DIVMTQSPLSLPVTPGEPASISCQPSQEVVHMNNVVYLHWYQQKPGQAPRLLIYKVSNRFPGVPDRFSGSGSGTDFTLKISRVEAEDVGVYYCAQGTSHPFTFGQGTKLEIK

SEQ ID NO: 145 - protein, 112 aa, synthetic construct
  REGION 1..112: note = an artificially synthesized sequence
DIVMTQSPLSLPVTPGEPASISCQPSQEVVHMNRNTYLHWYQQKPGQAPRLLIYKVSNVFPGVPDRFSGSGSGTDFTLKISRVEAEDVGVYYCAQGTHHPFTFGQGTKLEIK

SEQ ID NO: 146 - protein, 112 aa, synthetic construct
  REGION 1..112: note = an artificially synthesized sequence
DIVMTQSPLSLPVTPGEPASISCQPSEEVVHMNRNTYLHWYQQKPGQAPRLLIYKVSNLFPGVPDRFSGSGSGTDFTLKISRVEAEDVGVYYCAQGTHHPFTFGQGTKLEIK

SEQ ID NO: 147 - protein, 16 aa, synthetic construct
  REGION 1..16: note = an artificially synthesized sequence
QASQELVHMNRNTYLH

SEQ ID NO: 148 - protein, 16 aa, synthetic construct
  REGION 1..16: note = an artificially synthesized sequence
QPSQEVVHMNRNTYLH

SEQ ID NO: 149 - protein, 16 aa, synthetic construct
  REGION 1..16: note = an artificially synthesized sequence
QPSQEVVHMNNVVYLH

SEQ ID NO: 150 - protein, 16 aa, synthetic construct
  REGION 1..16: note = an artificially synthesized sequence
QPSQEVVHMNRNTYLH

SEQ ID NO: 151 - protein, 16 aa, synthetic construct
  REGION 1..16: note = an artificially synthesized sequence
QPSEEVVHMNRNTYLH

SEQ ID NO: 152 - protein, 7 aa, synthetic construct
  REGION 1..7: note = an artificially synthesized sequence
KVSNRFP

SEQ ID NO: 153 - protein, 7 aa, synthetic construct
  REGION 1..7: note = an artificially synthesized sequence
KVSNRFP

SEQ ID NO: 154 - protein, 7 aa, synthetic construct
  REGION 1..7: note = an artificially synthesized sequence
KVSNRFP

SEQ ID NO: 155 - protein, 7 aa, synthetic construct
  REGION 1..7: note = an artificially synthesized sequence
KVSNVFP

SEQ ID NO: 156 - protein, 7 aa, synthetic construct
  REGION 1..7: note = an artificially synthesized sequence
KVSNLFP

SEQ ID NO: 157 - protein, 9 aa, synthetic construct
  REGION 1..9: note = an artificially synthesized sequence
AQGTSVPFT

SEQ ID NO: 158 - protein, 9 aa, synthetic construct
  REGION 1..9: note = an artificially synthesized sequence
AQGTSHPFT

SEQ ID NO: 159 - protein, 9 aa, synthetic construct
  REGION 1..9: note = an artificially synthesized sequence
AQGTSHPFT

SEQ ID NO: 160 - protein, 9 aa, synthetic construct
  REGION 1..9: note = an artificially synthesized sequence
AQGTHHPFT

SEQ ID NO: 161 - protein, 9 aa, synthetic construct
  REGION 1..9: note = an artificially synthesized sequence
AQGTHHPFT

SEQ ID NO: 162 - protein, 122 aa, synthetic construct
  REGION 1..122: note = an artificially synthesized sequence
QVQLVESGGGVVQPGGSLRLSCAASGFTFSNAWMHWVRQAPGKGLEWVAQIKDKSQNYATYVAESVKGRFTISRADSKNSIYLQMNSLKTEDTAVYYCRYVHYAAGYGVDIWGQGTTVTVSS

SEQ ID NO: 163 - protein, 112 aa, synthetic construct
  REGION 1..112: note = an artificially synthesized sequence
DIVMTQSPLSLPVTPGEPASISCRSSQPLVHSNRNTYLHWYQQKPGQAPRLLIYKVSNRFSGVPDRFSGSGSGTDFTLKISRVEAEDVGVYYCGQGTQVPYTFGQGTKLEIK

SEQ ID NO: 164 - protein, 121 aa, synthetic construct [sequence omitted]

SEQ ID NO: 165 - protein, 109 aa, synthetic construct [sequence omitted]

SEQ ID NO: 166 - protein, 399 aa, synthetic construct
  REGION 1..399: note = an artificially synthesized sequence
LQDPCSNCPAGTFCDNNRNQICSPCPPNSFSSAGGQRTCDICRQCKGVFRTRKECSSTSNAECDCTPGFHCLGAGCSMCEQDCKQGQELTKKGCKDCCFGTFNDQKRGICRPWTNCSLDGKSVLVNGTKERDVVCGPSPADLSPGASSVTPPAPAREPGHSPQDIEGRMDPKSCDKTHTCPPCPAPELLGGPSVFLFPPKPKDTLMISRTPEVTCVVVDVSHEDPEVKFNWYVDGVEVHNAKTKPREEQYNSTYRVVSVLTVLHQDWLNGKEYKCKVSNKALPAPIEKTISKAKGQPREPQVYTLPPSREEMTKNQVSLTCLVKGFYPSDIAVEWESNGQPENNYKTTPPVLDSDGSFFLYSKLTVDKSRWQQGNVFSCSVMHEALHNHYTQKSLSLSP

SEQ ID NO: 167 - protein, 444 aa, synthetic construct
  REGION 1..444: note = an artificially synthesized sequence
EVQLVQSGAEVKKPGESLRISCKGSGYSFSTYWISWVRQMPGKGLEWMGKIYPGDSYTNYSPSFQGQVTISADKSISTAYLQWSSLKASDTAMYYCARGYGIFDYWGQGTLVTVSSASTKGPSVFPLAPSSKSTSGGTAALGCLVKDYFPEPVTVSWNSGALTSGVHTFPAVLQSSGLYSLSSVVTVPSSSLGTQTYICNVNHKPSNTKVDKKVEPKSCDKTHTCPPCPAPELLAGPSVFLFPPKPKDTLMISRTPEVTCVVVDVSFEDPEVKFNWYVDGVEVHNAKTKPREEPYNSTYRVVSVLTVLHQDWLNGKEYKCKVSNKAAPAPIEKTISKAKGQPREPQVYTLPPSRDELTKNQVSLTCLVKGFYPSDIAVEWESNGQPENNYKTTPPVLDSDGSFFLYSKLTVDKSRWQQGNVFSCSVMHEALHNHYTQKSLSLSP

SEQ ID NO: 168 - protein, 214 aa, synthetic construct
  REGION 1..214: note = an artificially synthesized sequence
SYELTQPPSVSVSPGQTASITCSGDNIGDQYAHWYQQKPGQSPVLVIYQDKNRPSGIPERFSGSNSGNTATLTISGTQAMDEADYYCATYTGFGSLAVFGGGTKLTVLGQPKAAPSVTLFPPSSEELQANKATLVCLISDFYPGAVTVAWKADSSPVKAGVETTTPSKQSNNKYAASSYLSLTPEQWKSHRSYSCQVTHEGSTVEKTVAPTECS

SEQ ID NO: 169 - protein, 212 aa, synthetic construct
  REGION 1..212: note = an artificially synthesized sequence
QDGNEEMGGITQTPYKVSISGTTVILTCPQYPGSEILWQHNDKNIGGDEDDKNIGSDEDHLSLKEFSELEQSGYYVCYPRGSKPEDANFYLYLRARVGSADDAKKDAAKKDDAKKDDAKKDGSQSIKGNHLVKVYDYQEDGSVLLTCDAEAKNITWFKDGKMIGFLTEDKKKWNLGSNAKDPRGMYQCKGSQNKSKPLQVYYRMDYKDDDDK

SEQ ID NO: 170 - protein, 207 aa, Homo sapiens
MQSGTHWRVLGLCLLSVGVWGQDGNEEMGGITQTPYKVSISGTTVILTCPQYPGSEILWQHNDKNIGGDEDDKNIGSDEDHLSLKEFSELEQSGYYVCYPRGSKPEDANFYLYLRARVCENCMEMDVMSVATIVIVDICITGGLLLLVYYWSKNRKAKAKPVTRGAGAGGRQRGQNKERPPPVPNPDYEPIRKGQRDLYSGLNQRRI

SEQ ID NO: 171 - protein, 4 aa, synthetic construct
  REGION 1..4: note = an artificially synthesized sequence
GGGS

SEQ ID NO: 172 - protein, 4 aa, synthetic construct
  REGION 1..4: note = an artificially synthesized sequence
SGGG

SEQ ID NO: 173 - protein, 5 aa, synthetic construct
  REGION 1..5: note = an artificially synthesized sequence
GGGGS

SEQ ID NO: 174 - protein, 5 aa, synthetic construct
  REGION 1..5: note = an artificially synthesized sequence
SGGGG

SEQ ID NO: 175 - protein, 6 aa, synthetic construct
  REGION 1..6: note = an artificially synthesized sequence
GGGGGS

SEQ ID NO: 176 - protein, 6 aa, synthetic construct
  REGION 1..6: note = an artificially synthesized sequence
SGGGGG

SEQ ID NO: 177 - protein, 7 aa, synthetic construct
  REGION 1..7: note = an artificially synthesized sequence
GGGGGGS

SEQ ID NO: 178 - protein, 7 aa, synthetic construct
  REGION 1..7: note = an artificially synthesized sequence
SGGGGGG

SEQ ID NO: 179 - protein, 189 aa, synthetic construct
  REGION 1..189: note = an artificially synthesized sequence
LQDPCSNCPAGTFCDNNRNQICSPCPPNSFSSAGGQRTCDICRQCKGVFRTRKECSSTSNAECDCTPGFHCLGAGCSMCEQDCKQGQELTKKGCKDCCFGTFNDQKRGICRPWTNCSLDGKSVLVNGTKERDVVCGPSPADLSPGASSVTPPAPAREPGHSPQHHHHHHGGGGSGLNDIFEAQKIEWHE

SEQ ID NO: 180 - protein, 22 aa, synthetic construct
  REGION 1..22: note = an artificially synthesized sequence
LQDPCSNCPAGTFCDNNRNQIC

SEQ ID NO: 181 - protein, 31 aa, synthetic construct
  REGION 1..31: note = an artificially synthesized sequence
DCTPGFHCLGAGCSMCEQDCKQGQELTKKGC

SEQ ID NO: 182 - protein, 72 aa, synthetic construct
  REGION 1..72: note = an artificially synthesized sequence
SPCPPNSFSSAGGQRTCDICRQCKGVFRTRKECSSTSNAECDCTPGFHCLGAGCSMCEQDCKQGQELTKKGC

SEQ ID NO: 183 - protein, 63 aa, synthetic construct
  REGION 1..63: note = an artificially synthesized sequence
LQDPCSNCPAGTFCDNNRNQICSPCPPNSFSSAGGQRTCDICRQCKGVFRTRKECSSTSNAEC

SEQ ID NO: 184 - protein, 122 aa, synthetic construct
  REGION 1..122: note = an artificially synthesized sequence
QVQLVESGGGVVQPGGSLRLSCAASGFTFSNAWMHWVRKAPGKGLEWVAQIKDKSQNYATYVAESVKGRFTISRADSKNSIYLQMNSLKTEDTAVYYCRYVHYAAGYGVDIWGQGTTVTVSS

SEQ ID NO: 185 - protein, 112 aa, synthetic construct
  REGION 1..112: note = an artificially synthesized sequence
DIVMTQSPLSLPVTPGEPASISCRSSQPLVHSNRNTYLHWYQEKPGQAPRLLIYKVSNRFSGVPDRFSGSGSGTDFTLKISRVEAEDVGVYYCGQGTQVPYTFGQGTKLEIK

SEQ ID NO: 186 - protein, 116 aa, synthetic construct
  REGION 1..116: note = an artificially synthesized sequence
QVQLQQSGPQLVRPGASVKISCKASGYSFTSYWMHWVNQRPGQGLEWIGMIDPSYSETRLNQKFKDKATLTVDKSSSTAYMQLSSPTSEDSAVYYCALYGNYFDYWGQGTTLTVSS

SEQ ID NO: 187 - protein, 107 aa, synthetic construct
  REGION 1..107: note = an artificially synthesized sequence
DIQMTQSSSSFSVSLGDRVTITCKASEDIYNRLAWYQQKPGNAPRLLISGATSLETGVPSRFSGSGSGKDYTLSITSLQTEDVATYYCQQYWSTPYTFGGGTKLEVK

SEQ ID NO: 188 - protein, 122 aa, synthetic construct; identical to SEQ ID NO: 162
  REGION 1..122: note = an artificially synthesized sequence

SEQ ID NO: 189 - protein, 112 aa, synthetic construct; identical to SEQ ID NO: 163
  REGION 1..112: note = an artificially synthesized sequence

SEQ ID NO: 190 - protein, 117 aa, synthetic construct
  REGION 1..117: note = an artificially synthesized sequence
EVQLQQSGPELVKPGASMKISCKASGYSFTGYTMNWVKQSHGKNLEWIGLINPYNGGTIYNQKFKGKATLTVDKSSSTAYMELLSLTSEDSAVYYCARDYGFVLDYWGQGTTLTVSS

SEQ ID NO: 191 - protein, 107 aa, synthetic construct
  REGION 1..107: note = an artificially synthesized sequence
DIVLTQSPSIMSVSPGEKVTITCSASSSVSYMHWFQQKPGTSPKLCIYSTSNLASGVPARFSGRGSGTSYSLTISRVAAEDAATYYCQQRSNYPPWTFGGGTKLEIK

SEQ ID NO: 192 - protein, 219 aa, synthetic construct
  REGION 1..219: note = an artificially synthesized sequence
DIVMTQSPLSLPVTPGEPASISCRSSQPLVHSNRNTYLHWYQEKPGQAPRLLIYKVSNRFSGVPDRFSGSGSGTDFTLKISRVEAEDVGVYYCGQGTQVPYTFGQGTKLEIKRTVAAPSVFIFPPSDEQLKSGTAEVVCLLNNFYPREAKVQWKVDNALQSGNSEESVTEQDSKDSTYSLSSTLELSKADYEKHKVYACEVTHQGLSSPVTKSFNRGEC

SEQ ID NO: 193 - protein, 447 aa, synthetic construct; identical to SEQ ID NO: 41
  REGION 1..447: note = an artificially synthesized sequence

SEQ ID NO: 194 - protein, 450 aa, synthetic construct
  REGION 1..450: note = an artificially synthesized sequence
QVQLVESGGGVVQPGGSLRLSCAASGFTFSNAWMHWVRKAPGKGLEWVAQIKDKSQNYATYVAESVKGRFTISRADSKNSIYLQMNSLKTEDTAVYYCRYVHYAAGYGVDIWGQGTTVTVSSASTKGPSVFPLAPSSKSTSGGTAALGCLVKDYFPEPVTVSWNSGALTSGVHTFPAVLKSSGLYSLSSVVTVPSSSLGTQTYICNVNHKPSNTKVDKRVEPKSCDKTHTCPPCPAPEAAGGPSVFLFPPKPKDTLMISRTPEVTCVVVDVSHEDPEVKFNWYVDGVEVHNAKTKPREEQYASTYRVVSVLTVLHQDWLNGKEYKCKVSNKALPAPIEKTISKAKGQPREPQVYTLPPSRKEMTKNQVSLTCLVKGFYPSDIAVEWESNGQPENNYKTTPPVLDSDGSFFLYSKLTVDKSRWQQGNVFSCSVMHEALHNHYTQKSLSLSP

SEQ ID NO: 195 - protein, 214 aa, synthetic construct; identical to SEQ ID NO: 50
  REGION 1..214: note = an artificially synthesized sequence

SEQ ID NO: 196 - protein, 220 aa, Homo sapiens
MASAGMQILGVVLTLLGWVNGLVSCALPMWKVTAFIGNSIVVAQVVWEGLWMSCVVQSTGQMQCKVYDSLLALPQDLQAARALCVIALLVALFGLLVYLAGAKCTTCVEEKDSKARLVLTSGIVFVISGVLTLIPVCWTAHAVIRDFYNPLVAEAQKRELGASLYLGWAASGLLLLGGGLLCCTCPSGGSQGPSHYMARYSTSAPAISRGPSEYPTKNYV

SEQ ID NO: 197 - protein, 220 aa, Homo sapiens
MASAGMQILGVVLTLLGWVNGLVSCALPMWKVTAFIGNSIVVAQVVWEGLWMSCVVQSTGQMQCKVYDSLLALPQDLQAARALCVIALLVALFGLLVYLAGAKCTTCVEEKDSKARLVLTSGIVFVISGVLTLIPVCWTAHAIIRDFYNPLVAEAQKRELGASLYLGWAASGLLLLGGGLLCCTCPSGGSQGPSHYMARYSTSAPAISRGPSEYPTKNYV

SEQ ID NO: 198 - protein, 217 aa, Homo sapiens
MASTGLELLGMTLAVLGWLGTLVSCALPLWKVTAFIGNSIVVAQVVWEGLWMSCVVQSTGQMQCKVYDSLLALPQDLQAARALCVIALLLALLGLLVAITGAQCTTCVEDEGAKARIVLTAGVILLLAGILVLIPVCWTAHAIIQDFYNPLVAEALKRELGASLYLGWAAAALLMLGGGLLCCTCPPPQVERPRGPRLGYSIPSRSGASGLDKRDYV

SEQ ID NO: 199 - protein, 220 aa, Homo sapiens
MSMGLEITGTALAVLGWLGTIVCCALPMWRVSAFIGSNIITSQNIWEGLWMNCVVQSTGQMQCKVYDSLLALPQDLQAARALIVVAILLAAFGLLVALVGAQCTNCVQDDTAKAKITIVAGVLFLLAALLTLVPVSWSANTIIRDFYNPVVPEAQKREMGAGLYVGWAAAALQLLGGALLCCSCPPREKKYTATKVVYSAPRSTGPGASLGTGYDRKDYV

SEQ ID NO: 200 - protein, 209 aa, Homo sapiens
MASMGLQVMGIALAVLGWLAVMLCCALPMWRVTAFIGSNIVTSQTIWEGLWMNCVVQSTGQMQCKVYDSLLALPQDLQAARALVIISIIVAALGVLLSVVGGKCTNCLEDESAKAKTMIVAGVVFLLAGLMVIVPVSWTAHNIIQDFYNPLVASGQKREMGASLYVGWAASGLLLLGGGLLCCNCPPRTDKPYSAKYSAARSAAASNYV

SEQ ID NO: 201 - protein, 219 aa, Mus musculus
MASTGLQILGIVLTLLGWVNALVSCALPMWKVTAFIGNSIVVAQMVWEGLWMSCVVQSTGQMQCKVYDSLLALPQDLQAARALCVVTLLIVLLGLLVYLAGAKCTTCVEDRNSKSRLVLISGIIFVISGVLTLIPVCWTAHSIIQDFYNPLVADAQKRELGASLYLGWAASGLLLLGGGLLCCACSSGGTQGPRHYMACYSTSVPHSRGPPEYPTKNYV

SEQ ID NO: 202 - protein, 217 aa, Mus musculus
MASTGLELLGMTLAVLGWLGTLVSCALPLWKVTAFIGNSIVVAQVVWEGLWMSCVVQSTGQMQCKVYDSLLALPQDLQAARALCVVALLLALLGLLVAITGAQCTTCVEDEGAKARIVLTAGVLLLLSGILVLIPVCWTAHAIIQDFYNPLVAEALKRELGASLYLGWAAAALLMLGGGLLCCTCPPSHFERPRGPRLGYSIPSRSGASGLDKRDYV

SEQ ID NO: 203 - protein, 219 aa, Mus musculus
MSMGLEITGTSLAVLGWLCTIVCCALPMWRVSAFIGSSIITAQITWEGLWMNCVVQSTGQMQCKMYDSLLALPQDLQAARALIVVSILLAAFGLLVALVGAQCTNCVQDETAKAKITIVAGVLFLLAALLTLVPVSWSANTIIRDFYNPLVPEAQKREMGAGLYVGWAAAALQLLGGALLCCSCPPRDKYAPTKILYSAPRSTGPGTGTGTAYDRKDYV

SEQ ID NO: 204 - protein, 210 aa, Mus musculus
MASMGLQVLGISLAVLGWLGIILSCALPMWRVTAFIGSNIVTAQTSWEGLWMNCVVQSTGQMQCKMYDSMLALPQDLQAARALMVISIIVGALGMLLSVVGGKCTNCMEDETVKAKIMITAGAVFIVASMLIMVPVSWTAHNVIRDFYNPMVASGQKREMGASLYVGWAASGLLLLGGGLLCCSCPPRSNDKPYSAKYSAARSVPASNYV

SEQ ID NO: 205 - protein, 220 aa, synthetic construct
  REGION 1..220: note = an artificially synthesized sequence
MASAGMQILGVVLTLLGWVNGLVSCALPMWKVTAFIGNSIVVAQVVWEGLWMSCVVQSTGQMQCKVYDSLLALPQDLQAARALCVIALLVALFGLLVYLAGAKCTTCVEEKDSKARLVLTSGIVFVISGVLTLIPVCWTAHAIIRDFYNPLVAEALKRELGASLYLGWAASGLLLLGGGLLCCTCPSGGSQGPSHYMARYSTSAPAISRGPSEYPTKNYV

SEQ ID NO: 206 - DNA, 20 bp, synthetic construct
  misc_feature 1..20: note = An artificially synthesized nucleotide sequence
  source 1..20: mol_type = other DNA
gggtggacgtcttatcagga

SEQ ID NO: 207 - DNA, 20 bp, synthetic construct
  misc_feature 1..20: note = An artificially synthesized nucleotide sequence
  source 1..20: mol_type = other DNA
gagctcctctcttcacccct

SEQ ID NO: 208 - DNA, 20 bp, synthetic construct
  misc_feature 1..20: note = An artificially synthesized nucleotide sequence
  source 1..20: mol_type = other DNA
gagtccactggcgtcttcac

SEQ ID NO: 209 - DNA, 23 bp, synthetic construct
  misc_feature 1..23: note = An artificially synthesized nucleotide sequence
  source 1..23: mol_type = other DNA
atcttgaggctgttgtcatactt

SEQ ID NO: 210 - protein, 443 aa, synthetic construct
QVQLVESGGGVVQPGGSLRLSCAASGFTFSSYTMSWVRQAPGQGLEWMGTISSGGGRTYYPDSVKGRFTISRDNSKNTLYLQMNSLRDEDTAVYYCARGDYRYDGFAYWGEGTLVTVSSAKTTPPSVYPLAPGSAAQTNSMVTLGCLVKGYFPEPVTVTWNSGSLSSGVHTFPAVLQSDLYTLSSSVTVPSSTWPSETVTCNVAHPASSTKVDKKIVPRDCGCKPCICTVKEVSKVFIFPPKPKDVLTITLTPKVTCVVVDISKDDPEVQFSWFVDDVEVHTAQTQPREEQFNSTFRSVSELPIMHQDWLNGKEFKCRVNSAAFPAPIEKTISKTKGRPKAPQVYTIPPPKEQMAKDKVSLTCMITDFFPEDITVEWQWNGQPAENYKNTQPIMDTDGSYFVYSKLNVQKSNWEAGNTFTCSVLHEGLHNHHTEKSLSHSPGK

SEQ ID NO: 211 - protein, 214 aa, synthetic construct
DIQMTQSPSSLSASVGDRVTITCRASYNIDSYLAWYQQKPGKAPELLIYYSTLLVDGVPDRFSGSRSGTDFTLTISSLQPEDFATYYCQHYYSIPYTFGQGTKVEIERADAAPTVSIFPPSSEQLTSGGASVVCFLNNFYPKDINVKWKIDGSERQNGVLNSWTDQDSKDSTYSMSSTLTLTKDEYERHNSYTCEATHKTSTSPIVKSFNRNEC

SEQ ID NO: 212 - DNA, 1329 bp, synthetic construct
  source 1..1329: mol_type = other DNA
caggtgcagctggtggagtctggaggaggagtggtgcagccaggaggatctctgaggctgagctgtgcagcatccggcttcacctttagctcctacaccatgtcttgggtgaggcaggcacctggacagggactggagtggatgggcacaatcagctccggcggcggcaggacctactatcctgacagcgtgaagggccggtttaccatctctagagacaacagcaagaatacactgtacctgcagatgaacagcctgagggacgaggatacagccgtgtactattgcgcaagaggcgactaccgctatgatggctttgcctattggggagagggcaccctggtgacagtgtcctctgccaaaacgacacccccatctgtctatccactggcccctggatctgctgcccaaactaactccatggtgaccctgggatgcctggtcaagggctatttccctgagccagtgacagtgacctggaactctggatccctgtccagcggtgtgcacaccttcccagctgtcctgcagtctgacctctacactctgagcagctcagtgactgtcccctccagcacctggcccagcgagaccgtcacctgcaacgttgcccacccggccagcagcaccaaggtggacaagaaaattgtgcccagggattgtggttgtaagccttgcatatgtacagtcaaagaagtatcaaaggtcttcatcttccccccaaagcccaaggatgtgctcaccattactctgactcctaaggtcacgtgtgttgtggtagacatcagcaaggatgatcccgaggtccagttcagctggtttgtagatgatgtggaggtgcacacagctcagacgcaaccccgggaggagcagttcaacagcactttccgctcagtcagtgaacttcccatcatgcaccaggactggctcaatggcaaggagttcaaatgcagggtcaacagtgcagctttccctgcccccatcgagaaaaccatctccaaaaccaaaggcagaccgaaggctccacaggtgtacaccattccacctcccaaggagcagatggccaaggataaagtcagtctgacctgcatgataacagacttcttccctgaagacattactgtggagtggcagtggaatgggcagccagcggagaactacaagaacactcagcccatcatggacacagatggctcttacttcgtctacagcaagctcaatgtgcagaagagcaactgggaggcaggaaatactttcacctgctctgtgttacatgagggcctgcacaaccaccatactgagaagagcctctcccactctcctggtaaa

SEQ ID NO: 213 - DNA, 642 bp, synthetic construct
  source 1..642: mol_type = other DNA
gacatccagatgacccagtcccctagctccctgtccgcctctgtgggcgacagggtgaccatcacatgccgggccagctacaacatcgattcctacctggcctggtatcagcagaagcccggcaaggcccctgagctgctgatctactactctacactgctggtggatggcgtgcccgaccggttcagcggatccagatctggcaccgactttaccctgacaatctctagcctgcagccagaggatttcgccacatactattgtcagcactactattctatcccctatacctttggccagggcacaaaggtggagatcgagcgagccgatgcggccccaactgtatccatcttcccaccatccagtgagcagttaacatctggaggtgcctcagtcgtgtgcttcttgaacaacttctaccccaaagacatcaatgtcaagtggaagattgatggcagtgaacgacaaaatggcgtcctgaacagttggactgatcaggacagcaaagacagcacctacagcatgagcagcaccctcacgttgaccaaggacgagtatgaacgacataacagctatacctgtgaggccactcacaagacatcaacttcacccattgtcaagagcttcaacaggaatgagtgt

SEQ ID NO: 214 - DNA, 18 bp, synthetic construct
  source 1..18: mol_type = other DNA
agtggttgagccgtggag

SEQ ID NO: 215 - DNA, 19 bp, synthetic construct
  source 1..19: mol_type = other DNA
cggtagtgaacccgttgat